European Patent Application EP 4 523 697 A1, published March 19, 2025. Title: THERAPEUTIC AGENT COMPRISING MULTISPECIFIC ANTIBODY AND USE THEREOF IN TUMOR THERAPY. Applicant: HANGZHOU VIROMAB BIOTECH CO., LTD. Application EP 23802842.7. The sequence listing filed with the application follows.

SEQUENCE LISTING (60 sequences)

SEQ ID NO: 1 - protein, 50 aa, synthetic construct
EQKLISEEDLGGGGSGGGGSEQKLISEEDLGGGGSGGGGSEQKLISEEDL

SEQ ID NO: 2 - protein, 47 aa, synthetic construct
YPYDVPDYAGGGGSGGGGSYPYDVPDYAGGGGSGGGGSYPYDVPDYA

SEQ ID NO: 3 - protein, 47 aa, synthetic construct
NWSHPQFEKGGGGSGGGGSNWSHPQFEKGGGGSGGGGSNWSHPQFEK

SEQ ID NO: 4 - protein, 64 aa, synthetic construct
EQKLISEEDLGEQKLISEEDLGEQKLISEEDLGGSYPYDVPDYAGYPYDVPDYAGYPYDVPDYA

SEQ ID NO: 5 - protein, 43 aa, synthetic construct
EQKLISEEDLGEQKLISEEDLGGSYPYDVPDYAGYPYDVPDYA

SEQ ID NO: 6 - protein, 55 aa, synthetic construct
FVPVFLPAKPTTTPAPRPPTPAPTIASQPLSLRPEACRPAAGGAVHTRGLDFACD

SEQ ID NO: 7 - protein, 28 aa, synthetic construct
IYIWAPLAGTCGVLLLSLVITLYCNHRN

SEQ ID NO: 8 - protein, 22 aa, synthetic construct
MLLLVTSLLLCELPHPAFLLIP

SEQ ID NO: 9 - protein, 117 aa, synthetic construct
TGTIETTGNISAEKGGSIILQCHLSSTTAQVTQVNWEQQDQLLAICNADLGWHISPSFKDRVAPGPGLGLTLQSLTVNDTGEYFCIYHTYPDGTYTGRIFLEVLESSVAEHGARFQI

SEQ ID NO: 10 - protein, 202 aa, synthetic construct
TGTIETTGNISAEKGGSIILQCHLSSTTAQVTQVNWEQQDQLLAICNADLGWHISPSFKDRVAPGPGLGLTLQSLTVNDTGEYFCIYHTYPDGTYTGRIFLEVLESSVAEHGARFQIASFVPVFLPAKPTTTPAPRPPTPAPTIASQPLSLRPEACRPAAGGAVHTRGLDFACDIYIWAPLAGTCGVLLLSLVITLYCNHRN

SEQ ID NO: 11 - protein, 145 aa, synthetic construct
EQKLISEEDLGGGGSGGGGSEQKLISEEDLGGGGSGGGGSEQKLISEEDLGGGGSGGGGSASFVPVFLPAKPTTTPAPRPPTPAPTIASQPLSLRPEACRPAAGGAVHTRGLDFACDIYIWAPLAGTCGVLLLSLVITLYCNHRN

SEQ ID NO: 12 - protein, 142 aa, synthetic construct
YPYDVPDYAGGGGSGGGGSYPYDVPDYAGGGGSGGGGSYPYDVPDYAGGGGSGGGGSASFVPVFLPAKPTTTPAPRPPTPAPTIASQPLSLRPEACRPAAGGAVHTRGLDFACDIYIWAPLAGTCGVLLLSLVITLYCNHRN

SEQ ID NO: 13 - protein, 142 aa, synthetic construct
NWSHPQFEKGGGGSGGGGSNWSHPQFEKGGGGSGGGGSNWSHPQFEKGGGGSGGGGSASFVPVFLPAKPTTTPAPRPPTPAPTIASQPLSLRPEACRPAAGGAVHTRGLDFACDIYIWAPLAGTCGVLLLSLVITLYCNHRN

SEQ ID NO: 14 - protein, 149 aa, synthetic construct
EQKLISEEDLGEQKLISEEDLGEQKLISEEDLGGSYPYDVPDYAGYPYDVPDYAGYPYDVPDYAASFVPVFLPAKPTTTPAPRPPTPAPTIASQPLSLRPEACRPAAGGAVHTRGLDFACDIYIWAPLAGTCGVLLLSLVITLYCNHRN

SEQ ID NO: 15 - protein, 246 aa, synthetic construct
EQKLISEEDLGEQKLISEEDLGGSYPYDVPDYAGYPYDVPDYAGTGTIETTGNISAEKGGSIILQCHLSSTTAQVTQVNWEQQDQLLAICNADLGWHISPSFKDRVAPGPGLGLTLQSLTVNDTGEYFCIYHTYPDGTYTGRIFLEVLESSVAEHGARFQIASFVPVFLPAKPTTTPAPRPPTPAPTIASQPLSLRPEACRPAAGGAVHTRGLDFACDIYIWAPLAGTCGVLLLSLVITLYCNHRN

SEQ ID NO: 16 - protein, 18 aa, synthetic construct
GSTSGSGKPGSGEGSTKG

SEQ ID NO: 17 - protein, 256 aa, synthetic construct
DIVLTQSPAFLAVSLGQRATISCRASESVDNYGFSFMNWFQQKPGQPPKLLIYAISNRGSGVPARFSGSGSGTDFSLNIHPVEEDDPAMYFCQQTKEVPWTFGGGTKLEIKGSTSGSGKPGSGEGSTKGQVQLQESGGDLVKPGGSLKLSCAASGFTFSHYGMSWVRQTPDKRLEWVATIGSRGTYTHYPDSVKGRFTISRDNDKNALYLQMNSLKSEDTAMYYCARRSEFYYYGNTYYYSAMDYWGQGASVTVSS

SEQ ID NO: 18 - protein, 15 aa, synthetic construct
GGGGSGGGGSGGGGS

SEQ ID NO: 19 - protein, 248 aa, synthetic construct
EVKLVESGGDLVKPGGSLKLSCAASGFTFSSYGMSWVRQTPDKRLEWVATISRGGSYTYYPDSVKGRFTISRDNAKNTLYLQMSSLKSEDTAMYYCARRETYDEKGFAYWGQGTTVTVSSGGGGSGGGGSGGGGSDIELTQSPSSLTVTAGEKVTMSCKSSQSLLNSGNQKNYLTWYQQKPGQPPKLLIYWASTRESGVPDRFTGSGSGRDFTLTISSVQAEDLAVYYCQNDNSHPLTFGAGTKLELK

SEQ ID NO: 20 - protein, 8 aa, synthetic construct
GYTFTNYY

SEQ ID NO: 21 - protein, 8 aa, synthetic construct
LNPNNGDT

SEQ ID NO: 22 - protein, 13 aa, synthetic construct
ARTGRYEENAMDY

SEQ ID NO: 23 - protein, 10 aa, synthetic construct
ESVDSYGKSF

SEQ ID NO: 24 - skipped

SEQ ID NO: 25 - protein, 9 aa, synthetic construct
QQNNEDPWT

SEQ ID NO: 26 - protein, 111 aa, synthetic construct
ELVMTQSPASLAVSLGQRATISCRASESVDSYGKSFMHWYQLKPGQPPKLLIYRASNLESGVPARFSGSGSRTDFTLTIDPVEADDAATYYCQQNNEDPWTFGGGTKLEIK

SEQ ID NO: 27 - protein, 120 aa, synthetic construct
EVQLEQSGPELVKPGASVKMSCKASGYTFTNYYMKWVKQSHGKSLEWIGDLNPNNGDTFYNQKFKGKATLTVDKSSNTAYMQLNSLTSEDSAVYYCARTGRYEENAMDYWGQGTSVTVSS

SEQ ID NO: 28 - protein, 249 aa, synthetic construct
ELVMTQSPASLAVSLGQRATISCRASESVDSYGKSFMHWYQLKPGQPPKLLIYRASNLESGVPARFSGSGSRTDFTLTIDPVEADDAATYYCQQNNEDPWTFGGGTKLEIKGSTSGSGKPGSGEGSTKGEVQLEQSGPELVKPGASVKMSCKASGYTFTNYYMKWVKQSHGKSLEWIGDLNPNNGDTFYNQKFKGKATLTVDKSSNTAYMQLNSLTSEDSAVYYCARTGRYEENAMDYWGQGTSVTVSS

SEQ ID NO: 29 - protein, 120 aa, synthetic construct
QVQLVQSGAEVKKPGASVKVSCKASGYTFTNYYMKWVKQAPGQRLEWMGDLNPNNGDTFYNQKFKGRVTITVDKSASTAYMELSSLRSEDTAVYYCARTGRYEENAMDYWGQGTLVTVSS

SEQ ID NO: 30 - protein, 120 aa, synthetic construct
QVQLVQSGAEVKKPGASVKVSCKASGYTFTNYYMKWVKQAPGQSLEWIGDLNPNNGDTFYNQKFKGRVTITVDKSASTAYMELNSLRSEDTAVYYCARTGRYEENAMDYWGQGTLVTVSS

SEQ ID NO: 31 - protein, 120 aa, synthetic construct
QVQLVQSGAEVKKPGASVKVSCKASGYTFTNYYMKWVKQAPGQSLEWIGDLNPNNGDTFYNQKFKGKATLTVDKSASTAYMELNSLRSEDTAVYYCARTGRYEENAMDYWGQGTLVTVSS

SEQ ID NO: 32 - protein, 111 aa, synthetic construct
DIVLTQSPASLAVSPGQRATITCRASESVDSYGKSFMHWYQQKPGQPPKLLIYRASNLESGVPARFSGSGSRTDFTLTINPVEANDTANYYCQQNNEDPWTFGQGTKLEIK

SEQ ID NO: 33 - protein, 111 aa, synthetic construct
DLVMTQSPASLAVSPGQRATITCRASESVDSYGKSFMHWYQQKPGQPPKLLIYRASNLESGVPARFSGSGSRTDFTLTINPVEANDTANYYCQQNNEDPWTFGQGTKLEIK

SEQ ID NO: 34 - protein, 111 aa, synthetic construct
DLVMTQSPASLAVSPGQRATITCRASESVDSYGKSFMHWYQLKPGQPPKLLIYRASNLESGVPARFSGSGSRTDFTLTINPVEANDTANYYCQQNNEDPWTFGQGTKLEIK

SEQ ID NO: 35 - protein, 8 aa, synthetic construct
GFTFNTYA

SEQ ID NO: 36 - protein, 10 aa, synthetic construct
IRSKYNNYAT

SEQ ID NO: 37 - protein, 16 aa, synthetic construct
VRHGNFGNSYVSWFAY

SEQ ID NO: 38 - protein, 9 aa, synthetic construct
TGAVTTSNY

SEQ ID NO: 39 - skipped

SEQ ID NO: 40 - protein, 9 aa, synthetic construct
ALWYSNLWV

SEQ ID NO: 41 - protein, 125 aa, synthetic construct
EVKLLESGGGLVQPKGSLKLSCAASGFTFNTYAMNWVRQAPGKGLEWVARIRSKYNNYATYYADSVKDRFTISRDDSQSILYLQMNNLKTEDTAMYYCVRHGNFGNSYVSWFAYWGQGTLVTVSA

SEQ ID NO: 42 - protein, 109 aa, synthetic construct
QAVVTQESALTTSPGETVTLTCRSSTGAVTTSNYANWVQEKPDHLFTGLIGGTNKRAPGVPARFSGSLIGDKAALTITGAQTEDEAIYFCALWYSNLWVFGGGTKLTVL

SEQ ID NO: 43 - protein, 125 aa, synthetic construct
EVQLVESGGGLVQPGGSLRLSCAASGFTFNTYAMNWVRQAPGKGLEWVARIRSKYNNYATYYADSVKDRFTISRDDSKNSLYLQMNSLKTEDTAVYYCVRHGNFGNSYVSWFAYWGQGTLVTVSA

SEQ ID NO: 44 - protein, 125 aa, synthetic construct
EVQLVESGGGLVQPGGSLRLSCAASGFTFNTYAMNWVRQAPGKGLEWVARIRSKYNNYATYYADSVKDRFTISRDDSKNILYLQMNSLKTEDTAVYYCVRHGNFGNSYVSWFAYWGQGTLVTVSA

SEQ ID NO: 45 - protein, 125 aa, synthetic construct
EVQLVESGGGLVQPGGSLRLSCAASGFTFNTYAMNWVRQAPGKGLEWVARIRSKYNNYATYYADSVKDRFTISRDDSKNILYLQMNSLKTEDTAMYYCVRHGNFGNSYVSWFAYWGQGTLVTVSA

SEQ ID NO: 46 - protein, 109 aa, synthetic construct
QAVVTQEPSLTVSPGGTVTLTCRSSTGAVTTSNYANWVQQKPGQAPRGLIGGTNKRAPWTPARFSGSLLGGKAALTLSGAQPEDEAEYYCALWYSNLWVFGGGTKLTVL

SEQ ID NO: 47 - protein, 109 aa, synthetic construct
QAVVTQEPSLTVSPGGTVTLTCRSSTGAVTTSNYANWVQQKPGQAPRGLIGGTNKRAPWTPARFSGSLLGGKAALTLSGAQTEDEAEYYCALWYSNLWVFGGGTKLTVL

SEQ ID NO: 48 - protein, 109 aa, synthetic construct
QAVVTQEPSLTVSPGGTVTLTCRSSTGAVTTSNYANWVQQKPGQAPRGLIGGTNKRAPWTPARFSGSLLGGKAALTITGAQTEDEAEYYCALWYSNLWVFGGGTKLTVL

SEQ ID NO: 49 - protein, 109 aa, synthetic construct
QAVVTQEPSLTVSPGGTVTLTCRSSTGAVTTSNYANWVQQKPGQAPRGLIGGTNKRAPWVPARFSGSLLGDKAALTLSGAQTEDEAEYYCALWYSNLWVFGGGTKLTVL

SEQ ID NO: 50 - protein, 109 aa, synthetic construct
QAVVTQEPSLTVSPGGTVTLTCRSSTGAVTTSNYANWVQEKPGQAPRGLIGGTNKRAPWVPARFSGSLLGDKAALTLSGAQTEDEAEYYCALWYSNLWVFGGGTKLTVL

SEQ ID NO: 51 - protein, 109 aa, synthetic construct
QAVVTQEPSLTVSPGGTVTLTCRSSTGAVTTSNYANWVQQKPGQAPRTLIGGTNKRAPWTPARFSGSLLGGKAALTLSGAQPEDEAEYYCALWYSNLWVFGGGTKLTVL

SEQ ID NO: 52 - protein, 109 aa, synthetic construct
QAVVTQEPSLTVSPGGTVTLTCRSSTGAVTTSNYANWVQQKPGQAPRTLIGGTNKRAPWVPARFSGSLLGDKAALTLSGAQPEDEAEYYCALWYSNLWVFGGGTKLTVL

SEQ ID NO: 53 - protein, 109 aa, synthetic construct
QAVVTQEPSLTVSPGGTVTLTCRSSTGAVTTSNYANWVQEKPGQAPRTLIGGTNKRAPWVPARFSGSLLGDKAALTLSGAQPEDEAEYYCALWYSNLWVFGGGTKLTVL

SEQ ID NO: 54 - protein, 330 aa, synthetic construct
ASTKGPSVFPLAPSSKSTSGGTAALGCLVKDYFPEPVTVSWNSGALTSGVHTFPAVLQSSGLYSLSSVVTVPSSSLGTQTYICNVNHKPSNTKVDKRVEPKSCDKTHTCPPCPAPEFEGGPSVFLFPPKPKDTLMISRTPEVTCVVVDVSHEDPEVKFNWYVDGVEVHNAKTKPREEQYNSTYRVVSVLTVLHQDWLNGKEYKCKVSNKALPASIEKTISKAKGQPREPQVYTLPPSREEMTKNQVSLTCLVKGFYPSDIAVEWESNGQPENNYKTTPPVLDSDGSFFLYSKLTVDKSRWQQGNVFSCSVMHEALHNHYTQKSLSLSPGK

SEQ ID NO: 55 - protein, 107 aa, synthetic construct [sequence omitted]

SEQ ID NO: 56 - protein, 220 aa, synthetic construct
PCPAPEFEGGPSVFLFPPKPKDTLMISRTPEVTCVVVDVSHEDPEVKFNWYVDGVEVHNAKTKPREEQYNSTYRVVSVLTVLHQDWLNGKEYKCKVSNKALPASIEKTISKAKGQPREPQVYTLPPSREEMTKNQVSLTCLVKGFYPSDIAVEWESNGQPENNYKTTPPVLDSDGSFFLYSKLTVDKSRWQQGNVFSCSVMHEALHNHYTQKSLSLSPGK

SEQ ID NO: 57 - protein, 330 aa, synthetic construct [sequence omitted]

SEQ ID NO: 58 - protein, 8 aa, synthetic construct
WSHPQFEK

SEQ ID NO: 59 - protein, 9 aa, synthetic construct
NWSHPQFEK

SEQ ID NO: 60 - protein, 9 aa, synthetic construct
AWRHPQFGG